European Patent Specification EP 3 906 066 B1, published November 1, 2023. Title: GENE THERAPY CONSTRUCTS FOR TREATING WILSON DISEASE. Applicant: ULTRAGENYX PHARMACEUTICAL INC. The sequence listing filed with the application follows.

SEQUENCE LISTING (15 sequences)

SEQ ID NO: 1 - DNA, 3603 bp, Artificial Sequence
  Description of artificial sequence: Del 1-3 ATP7B, native
  misc_feature (223)..(225): Nucleotides 223-225 encode for serine residue S340 (numbering based on wild-type protein sequence)
  misc_feature (226)..(228): Nucleotides 226-228 encode for serine residue S341 (numbering based on wild-type protein sequence)
atgcctgagcaggagagacagatcacagccagagaaggggccagtcggaaaatcttatctaagctttctttgcctacccgtgcctgggaaccagcaatgaagaagagttttgcttttgacaatgttggctatgaaggtggtctggatggcctgggcccttcttctcaggtggccaccagcacagtcagggatggagccgaagggagtgggacagatcacaggtcttccagttctcattcccctggctccccaccgagaaaccaggtccagggcacatgcagtaccactctgattgccattgccggcatgacctgtgcatcctgtgtccattccattgaaggcatgatctcccaactggaaggggtgcagcaaatatcggtgtctttggccgaagggactgcaacagttctttataatccctctgtaattagcccagaagaactcagagctgctatagaagacatgggatttgaggcttcagtcgtttctgaaagctgttctactaaccctcttggaaaccacagtgctgggaattccatggtgcaaactacagatggtacacctacatctgtgcaggaagtggctccccacactgggaggctccctgcaaaccatgccccggacatcttggcaaagtccccacaatcaaccagagcagtggcaccgcagaagtgcttcttacagatcaaaggcatgacctgtgcatcctgtgtgtctaacatagaaaggaatctgcagaaagaagctggtgttctctccgtgttggttgccttgatggcaggaaaggcagagatcaagtatgacccagaggtcatccagcccctcgagatagctcagttcatccaggacctgggttttgaggcagcagtcatggaggactacgcaggctccgatggcaacattgagctgacaatcacagggatgacctgcgcgtcctgtgtccacaacatagagtccaaactcacgaggacaaatggcatcacttatgcctccgttgcccttgccaccagcaaagcccttgttaagtttgacccggaaattatcggtccacgggatattatcaaaattattgaggaaattggctttcatgcttccctggcccagagaaaccccaacgctcatcacttggaccacaagatggaaataaagcagtggaagaagtctttcctgtgcagcctggtgtttggcatccctgtcatggccttaatgatctatatgctgatacccagcaacgagccccaccagtccatggtcctggaccacaacatcattccaggactgtccattctaaatctcatcttctttatcttgtgtacctttgtccagctcctcggtgggtggtacttctacgttcaggcctacaaatctctgagacacaggtcagccaacatggacgtgctcatcgtcctggccacaagcattgcttatgtttattctctggtcatcctggtggttgctgtggctgagaaggcggagaggagccctgtgacattcttcgacacgccccccatgctctttgtgttcattgccctgggccggtggctggaacacttggcaaagagcaaaacctcagaagccctggctaaactcatgtctctccaagccacagaagccaccgttgtgacccttggtgaggacaatttaatcatcagggaggagcaagtccccatggagctggtgcagcggggcgatatcgtcaaggtggtccctgggggaaagtttccagtggatgggaaagtcctggaaggcaataccatggctgatgagtccctcatcacaggagaagccatgccagtcactaagaaacccggaagcactgtaattgcggggtctataaatgcacatggctctgtgctcattaaagctacccacgtgggcaatgacaccactttggctcagattgtgaaactggtggaagaggctcagatgtcaaaggcacccattcagcagctggctgaccggtttagtggatattttgtcccatttatcatcatcatgtcaactttgacgttggtggtatggattgtaatcggttttatcgattttggtgttgttcagagatactttcctaaccccaacaagcacatctcccagacagaggtgatcatccggtttgctttccagacgtccatcacggtgctgtgcattgcctgcccctgctccctggggctggccacgcccacggctgtcatggtgggcaccggggtggccgcgcagaacggcatcctcatcaagggaggcaagcccctggagatggcgcacaagataaagactgtgatgtttgacaagactggcaccattacccatggcgtccccagggtcatgcgggtgctcctgctgggggatgtggccacactgcccctcaggaaggttctggctgtggtggggactgcggaggccagcagtgaacaccccttgggcgtggcagtcaccaaatactgtaaagaggaacttggaacagagaccttgggatactgcacggacttccaggcagtgccaggctgtggaattgggtgcaaagtcagcaacgtggaaggcatcctggcccacagtgagcgccctttgagtgcaccggccagtcacctgaatgaggctggcagccttcccgcagaaaaagatgcagtcccccagaccttctctgtgctgattggaaaccgtgagtggctgaggcgcaacggtttaaccatttctagcgatgtcagtgacgctatgacagaccacgagatgaaaggacagacagccatcctggtggctattgacggtgtgctctgtgggatgatcgcaatcgcagacgctgtcaagcaggaggctgccctggctgtgcacacgctgcagagcatgggtgtggacgtggttctgatcacgggggacaaccggaagacagccagagctattgccacccaggttggcatcaacaaagtctttgcagaggtgctgccttcgcacaaggtggccaaggtccaggagctccagaataaagggaagaaagtcgccatggtgggggatggggtcaatgactccccggccttggcccaggcagacatgggtgtggccattggcaccggcacggatgtggccatcgaggcagccgacgtcgtccttatcagaaatgatttgctggatgtggtggctagcattcacctttccaagaggactgtccgaaggatacgcatcaacctggtcctggcactgatttataacctggttgggatacccattgcagcaggtgtcttcatgcccatcggcattgtgctgcagccctggatgggctcagcggccatggcagcctcctctgtgtctgtggtgctctcatccctgcagctcaagtgctataagaagcctgacctggagaggtatgaggcacaggcgcatggccacatgaagcccctgacggcatcccaggtcagtgtgcacataggcatggatgacaggtggcgggactcccccagggccacaccatgggaccaggtcagctatgtcagccaggtgtcgctgtcctccctgacgtccgacaagccatctcggcacagcgctgcagcagacgatgatggggacaagtggtctctgctcctgaatggcagggatgaggagcagtacatctga

SEQ ID NO: 2 - DNA, 145 bp, Artificial Sequence
  Description of artificial sequence: AAV2 ITR
ttggccactccctctctgcgcgctcgctcgctcactgaggccgggcgaccaaaggtcgcccgacgcccgggctttgcccgggcggcctcagtgagcgagcgagcgcgcagagagggagtggccaactccatcactaggggttcct

SEQ ID NO: 3 - DNA, 100 bp, Artificial Sequence
  Description of artificial sequence: enTTR Enhancer sequence
ctacctcgtgatcgcccggcccctgttcaaacatgtcctaatactctgtctctgcaagggtcatcagtagttttccatcttactcaacatcctcccagtg

SEQ ID NO: 4 - DNA, 95 bp, Artificial Sequence
  Description of artificial sequence: SV40 Small T Intron
gctctaaggtaaatataaaatttttaagtgtataatgtgttaaactactgattctaattgtttctctcttttagattccaacctttggaactgat

SEQ ID NO: 5 - DNA, 315 bp, Artificial Sequence
  Description of artificial sequence: rHBB Intron
gtgagcgggcgggacggcccttctcctccgggctgtaattagcgcttggtttaatgacggcttgtttcttttctgtggctgcgtgaaagccttgaggggctccgggagggccctttgtgcggggggagcggctcggggctgtccgcggggggacggctgccttcgggggggacggggcagggcggggttcggcttctggcgtgtgaccggcggctcaagagcctctgctaaccatgttcatgccttcttctttttcctacagctcctgggcaacgtgctggttattgtgctgtctcatcattttggcaaagaatt

SEQ ID NO: 6 - DNA, 215 bp, Artificial Sequence
  Description of artificial sequence: BGH polyadenylation signal sequence
gcctcgactgtgccttctagttgccagccatctgttgtttgcccctcccccgtgccttccttgaccctggaaggtgccactcccactgtcctttcctaataaaatgaggaaattgcatcgcattgtctgagtaggtgtcattctattctggggggtggggtggggcaggacagcaagggggaggattgggaagacaatagcaggcatgctgggga

SEQ ID NO: 7 - DNA, 198 bp, Artificial Sequence
  Description of artificial sequence: SV40 polyadenylation signal sequence
gatccagacatgataagatacattgatgagtttggacaaaccacaactagaatgcagtgaaaaaaatgctttatttgtgaaatttgtgatgctattgctttatttgtaaccattataagctgcaataaacaagttaacaacaacaattgcattcattttatgtttcaggttcagggggaggtgtgggaggttttttag

SEQ ID NO: 8 - protein, 1200 aa, Artificial Sequence
  Description of artificial sequence: DEL 1-3 ATP7B Native, protein
  MISC_FEATURE (75)..(75): Amino acid residue at position 75 corresponds to Serine S340 (numbering based on wild-type protein sequence)
  MISC_FEATURE (76)..(76): Amino acid residue at position 76 corresponds to Serine S341 (numbering based on wild-type protein sequence)
MPEQERQITAREGASRKILSKLSLPTRAWEPAMKKSFAFDNVGYEGGLDGLGPSSQVATSTVRDGAEGSGTDHRSSSSHSPGSPPRNQVQGTCSTTLIAIAGMTCASCVHSIEGMISQLEGVQQISVSLAEGTATVLYNPSVISPEELRAAIEDMGFEASVVSESCSTNPLGNHSAGNSMVQTTDGTPTSVQEVAPHTGRLPANHAPDILAKSPQSTRAVAPQKCFLQIKGMTCASCVSNIERNLQKEAGVLSVLVALMAGKAEIKYDPEVIQPLEIAQFIQDLGFEAAVMEDYAGSDGNIELTITGMTCASCVHNIESKLTRTNGITYASVALATSKALVKFDPEIIGPRDIIKIIEEIGFHASLAQRNPNAHHLDHKMEIKQWKKSFLCSLVFGIPVMALMIYMLIPSNEPHQSMVLDHNIIPGLSILNLIFFILCTFVQLLGGWYFYVQAYKSLRHRSANMDVLIVLATSIAYVYSLVILVVAVAEKAERSPVTFFDTPPMLFVFIALGRWLEHLAKSKTSEALAKLMSLQATEATVVTLGEDNLIIREEQVPMELVQRGDIVKVVPGGKFPVDGKVLEGNTMADESLITGEAMPVTKKPGSTVIAGSINAHGSVLIKATHVGNDTTLAQIVKLVEEAQMSKAPIQQLADRFSGYFVPFIIIMSTLTLVVWIVIGFIDFGVVQRYFPNPNKHISQTEVIIRFAFQTSITVLCIACPCSLGLATPTAVMVGTGVAAQNGILIKGGKPLEMAHKIKTVMFDKTGTITHGVPRVMRVLLLGDVATLPLRKVLAVVGTAEASSEHPLGVAVTKYCKEELGTETLGYCTDFQAVPGCGIGCKVSNVEGILAHSERPLSAPASHLNEAGSLPAEKDAVPQTFSVLIGNREWLRRNGLTISSDVSDAMTDHEMKGQTAILVAIDGVLCGMIAIADAVKQEAALAVHTLQSMGVDVVLITGDNRKTARAIATQVGINKVFAEVLPSHKVAKVQELQNKGKKVAMVGDGVNDSPALAQADMGVAIGTGTDVAIEAADVVLIRNDLLDVVASIHLSKRTVRRIRINLVLALIYNLVGIPIAAGVFMPIGIVLQPWMGSAAMAASSVSVVLSSLQLKCYKKPDLERYEAQAHGHMKPLTASQVSVHIGMDDRWRDSPRATPWDQVSYVSQVSLSSLTSDKPSRHSAAADDDGDKWSLLLNGRDEEQYI

SEQ ID NO: 9 - DNA, 2211 bp, Artificial Sequence
  Description of artificial sequence: Nucleic acid sequence encoding AAV9 capsid protein VP1
atggctgccgatggttatcttccagattggctcgaggacaaccttagtgaaggaattcgcgagtggtgggctttgaaacctggagcccctcaacccaaggcaaatcaacaacatcaagacaacgctcgaggtcttgtgcttccgggttacaaataccttggacccggcaacggactcgacaagggggagccggtcaacgcagcagacgcggcggccctcgagcacgacaaggcctacgaccagcagctcaaggccggagacaacccgtacctcaagtacaaccacgccgacgccgagttccaggagcggctcaaagaagatacgtcttttgggggcaacctcgggcgagcagtcttccaggccaaaaagaggcttcttgaacctcttggtctggttgaggaagcggctaagacggctcctggaaagaagaggcctgtagagcagtctcctcaggaaccggactcctccgcgggtattggcaaatcgggtgcacagcccgctaaaaagagactcaatttcggtcagactggcgacacagagtcagtcccagaccctcaaccaatcggagaacctcccgcagccccctcaggtgtgggatctcttacaatggcttcaggtggtggcgcaccagtggcagacaataacgaaggtgccgatggagtgggtagttcctcgggaaattggcattgcgattcccaatggctgggggacagagtcatcaccaccagcacccgaacctgggccctgcccacctacaacaatcacctctacaagcaaatctccaacagcacatctggaggatcttcaaatgacaacgcctacttcggctacagcaccccctgggggtattttgacttcaacagattccactgccacttctcaccacgtgactggcagcgactcatcaacaacaactggggattccggcctaagcgactcaacttcaagctcttcaacattcaggtcaaagaggttacggacaacaatggagtcaagaccatcgccaataaccttaccagcacggtccaggtcttcacggactcagactatcagctcccgtacgtgctcgggtcggctcacgagggctgcctcccgccgttcccagcggacgttttcatgattcctcagtacgggtatctgacgcttaatgatggaagccaggccgtgggtcgttcgtccttttactgcctggaatatttcccgtcgcaaatgctaagaacgggtaacaacttccagttcagctacgagtttgagaacgtacctttccatagcagctacgctcacagccaaagcctggaccgactaatgaatccactcatcgaccaatacttgtactatctctcaaagactattaacggttctggacagaatcaacaaacgctaaaattcagtgtggccggacccagcaacatggctgtccagggaagaaactacatacctggacccagctaccgacaacaacgtgtctcaaccactgtgactcaaaacaacaacagcgaatttgcttggcctggagcttcttcttgggctctcaatggacgtaatagcttgatgaatcctggacctgctatggccagccacaaagaaggagaggaccgtttctttcctttgtctggatctttaatttttggcaaacaaggaactggaagagacaacgtggatgcggacaaagtcatgataaccaacgaagaagaaattaaaactactaacccggtagcaacggagtcctatggacaagtggccacaaaccaccagagtgcccaagcacaggcgcagaccggctgggttcaaaaccaaggaatacttccgggtatggtttggcaggacagagatgtgtacctgcaaggacccatttgggccaaaattcctcacacggacggcaactttcacccttctccgctgatgggagggtttggaatgaagcacccgcctcctcagatcctcatcaaaaacacacctgtacctgcggatcctccaacggccttcaacaaggacaagctgaactctttcatcacccagtattctactggccaagtcagcgtggagatcgagtgggagctgcagaaggaaaacagcaagcgctggaacccggagatccagtacacttccaactattacaagtctaataatgttgaatttgctgttaatactgaaggtgtatatagtgaaccccgccccattggcaccagatacctgactcgtaatctgtaa

SEQ ID NO: 10 - protein, 736 aa, Artificial Sequence
  Description of artificial sequence: Amino acid sequence encoding AAV9 capsid protein VP1
MAADGYLPDWLEDNLSEGIREWWALKPGAPQPKANQQHQDNARGLVLPGYKYLGPGNGLDKGEPVNAADAAALEHDKAYDQQLKAGDNPYLKYNHADAEFQERLKEDTSFGGNLGRAVFQAKKRLLEPLGLVEEAAKTAPGKKRPVEQSPQEPDSSAGIGKSGAQPAKKRLNFGQTGDTESVPDPQPIGEPPAAPSGVGSLTMASGGGAPVADNNEGADGVGSSSGNWHCDSQWLGDRVITTSTRTWALPTYNNHLYKQISNSTSGGSSNDNAYFGYSTPWGYFDFNRFHCHFSPRDWQRLINNNWGFRPKRLNFKLFNIQVKEVTDNNGVKTIANNLTSTVQVFTDSDYQLPYVLGSAHEGCLPPFPADVFMIPQYGYLTLNDGSQAVGRSSFYCLEYFPSQMLRTGNNFQFSYEFENVPFHSSYAHSQSLDRLMNPLIDQYLYYLSKTINGSGQNQQTLKFSVAGPSNMAVQGRNYIPGPSYRQQRVSTTVTQNNNSEFAWPGASSWALNGRNSLMNPGPAMASHKEGEDRFFPLSGSLIFGKQGTGRDNVDADKVMITNEEEIKTTNPVATESYGQVATNHQSAQAQAQTGWVQNQGILPGMVWQDRDVYLQGPIWAKIPHTDGNFHPSPLMGGFGMKHPPPQILIKNTPVPADPPTAFNKDKLNSFITQYSTGQVSVEIEWELQKENSKRWNPEIQYTSNYYKSNNVEFAVNTEGVYSEPRPIGTRYLTRNL

SEQ ID NO: 11 - DNA, 6 bp, Artificial Sequence
  Description of artificial sequence: Consensus Kozak Sequence
gccgcc

SEQ ID NO: 12 - DNA, 190 bp, Artificial Sequence
  Description of artificial sequence: TTR promoter Sequence
atttcatagaacgaatgttccgatgctctaatctctctagacaaggttcatatttgtatgggttacttattctctctttgttgactaagtcaataatcagaatcagcaggtttgcagtcagattggcagggataagcagcctagctcaggagaagtgagtataaaagccccaggctgggagcagccatca

SEQ ID NO: 13 - protein, 1120 aa, Artificial Sequence
  Description of artificial sequence: DEL 1-4 ATP7B Native, protein
MPEQERQITAREGASRKILSKLSLPTRAWEPAMKKSFAFDNVGYEGGLDGLGPSSQVATSTVRSPEELRAAIEDMGFEASVVSESCSTNPLGNHSAGNSMVQTTDGTPTSVQEVAPHTGRLPANHAPDILAKSPQSTRAVAPQKCFLQIKGMTCASCVSNIERNLQKEAGVLSVLVALMAGKAEIKYDPEVIQPLEIAQFIQDLGFEAAVMEDYAGSDGNIELTITGMTCASCVHNIESKLTRTNGITYASVALATSKALVKFDPEIIGPRDIIKIIEEIGFHASLAQRNPNAHHLDHKMEIKQWKKSFLCSLVFGIPVMALMIYMLIPSNEPHQSMVLDHNIIPGLSILNLIFFILCTFVQLLGGWYFYVQAYKSLRHRSANMDVLIVLATSIAYVYSLVILVVAVAEKAERSPVTFFDTPPMLFVFIALGRWLEHLAKSKTSEALAKLMSLQATEATVVTLGEDNLIIREEQVPMELVQRGDIVKVVPGGKFPVDGKVLEGNTMADESLITGEAMPVTKKPGSTVIAGSINAHGSVLIKATHVGNDTTLAQIVKLVEEAQMSKAPIQQLADRFSGYFVPFIIIMSTLTLVVWIVIGFIDFGVVQRYFPNPNKHISQTEVIIRFAFQTSITVLCIACPCSLGLATPTAVMVGTGVAAQNGILIKGGKPLEMAHKIKTVMFDKTGTITHGVPRVMRVLLLGDVATLPLRKVLAVVGTAEASSEHPLGVAVTKYCKEELGTETLGYCTDFQAVPGCGIGCKVSNVEGILAHSERPLSAPASHLNEAGSLPAEKDAVPQTFSVLIGNREWLRRNGLTISSDVSDAMTDHEMKGQTAILVAIDGVLCGMIAIADAVKQEAALAVHTLQSMGVDVVLITGDNRKTARAIATQVGINKVFAEVLPSHKVAKVQELQNKGKKVAMVGDGVNDSPALAQADMGVAIGTGTDVAIEAADVVLIRNDLLDVVASIHLSKRTVRRIRINLVLALIYNLVGIPIAAGVFMPIGIVLQPWMGSAAMAASSVSVVLSSLQLKCYKKPDLERYEAQAHGHMKPLTASQVSVHIGMDDRWRDSPRATPWDQVSYVSQVSLSSLTSDKPSRHSAAADDDGDKWSLLLNGRDEEQYI

SEQ ID NO: 14 - DNA, 4485 bp, Artificial Sequence
  Description of artificial sequence: Expression cassette of exemplary vector DTC319
ttggccactccctctctgcgcgctcgctcgctcactgaggccgggcgaccaaaggtcgcccgacgcccgggctttgcccgggcggcctcagtgagcgagcgagcgcgcagagagggagtggccaactccatcactaggggttcctctacctcgtgatcgcccggcccctgttcaaacatgtcctaatactctgtctctgcaagggtcatcagtagttttccatcttactcaacatcctcccagtgatttcatagaacgaatgttccgatgctctaatctctctagacaaggttcatatttgtatgggttacttattctctctttgttgactaagtcaataatcagaatcagcaggtttgcagtcagattggcagggataagcagcctagctcaggagaagtgagtataaaagccccaggctgggagcagccatcagctctaaggtaaatataaaatttttaagtgtataatgtgttaaactactgattctaattgtttctctcttttagattccaacctttggaactgatgccgccaccatgcctgagcaggagagacagatcacagccagagaaggggccagtcggaaaatcttatctaagctttctttgcctacccgtgcctgggaaccagcaatgaagaagagttttgcttttgacaatgttggctatgaaggtggtctggatggcctgggcccttcttctcaggtggccaccagcacagtcagggatggagccgaagggagtgggacagatcacaggtcttccagttctcattcccctggctccccaccgagaaaccaggtccagggcacatgcagtaccactctgattgccattgccggcatgacctgtgcatcctgtgtccattccattgaaggcatgatctcccaactggaaggggtgcagcaaatatcggtgtctttggccgaagggactgcaacagttctttataatccctctgtaattagcccagaagaactcagagctgctatagaagacatgggatttgaggcttcagtcgtttctgaaagctgttctactaaccctcttggaaaccacagtgctgggaattccatggtgcaaactacagatggtacacctacatctgtgcaggaagtggctccccacactgggaggctccctgcaaaccatgccccggacatcttggcaaagtccccacaatcaaccagagcagtggcaccgcagaagtgcttcttacagatcaaaggcatgacctgtgcatcctgtgtgtctaacatagaaaggaatctgcagaaagaagctggtgttctctccgtgttggttgccttgatggcaggaaaggcagagatcaagtatgacccagaggtcatccagcccctcgagatagctcagttcatccaggacctgggttttgaggcagcagtcatggaggactacgcaggctccgatggcaacattgagctgacaatcacagggatgacctgcgcgtcctgtgtccacaacatagagtccaaactcacgaggacaaatggcatcacttatgcctccgttgcccttgccaccagcaaagcccttgttaagtttgacccggaaattatcggtccacgggatattatcaaaattattgaggaaattggctttcatgcttccctggcccagagaaaccccaacgctcatcacttggaccacaagatggaaataaagcagtggaagaagtctttcctgtgcagcctggtgtttggcatccctgtcatggccttaatgatctatatgctgatacccagcaacgagccccaccagtccatggtcctggaccacaacatcattccaggactgtccattctaaatctcatcttctttatcttgtgtacctttgtccagctcctcggtgggtggtacttctacgttcaggcctacaaatctctgagacacaggtcagccaacatggacgtgctcatcgtcctggccacaagcattgcttatgtttattctctggtcatcctggtggttgctgtggctgagaaggcggagaggagccctgtgacattcttcgacacgccccccatgctctttgtgttcattgccctgggccggtggctggaacacttggcaaagagcaaaacctcagaagccctggctaaactcatgtctctccaagccacagaagccaccgttgtgacccttggtgaggacaatttaatcatcagggaggagcaagtccccatggagctggtgcagcggggcgatatcgtcaaggtggtccctgggggaaagtttccagtggatgggaaagtcctggaaggcaataccatggctgatgagtccctcatcacaggagaagccatgccagtcactaagaaacccggaagcactgtaattgcggggtctataaatgcacatggctctgtgctcattaaagctacccacgtgggcaatgacaccactttggctcagattgtgaaactggtggaagaggctcagatgtcaaaggcacccattcagcagctggctgaccggtttagtggatattttgtcccatttatcatcatcatgtcaactttgacgttggtggtatggattgtaatcggttttatcgattttggtgttgttcagagatactttcctaaccccaacaagcacatctcccagacagaggtgatcatccggtttgctttccagacgtccatcacggtgctgtgcattgcctgcccctgctccctggggctggccacgcccacggctgtcatggtgggcaccggggtggccgcgcagaacggcatcctcatcaagggaggcaagcccctggagatggcgcacaagataaagactgtgatgtttgacaagactggcaccattacccatggcgtccccagggtcatgcgggtgctcctgctgggggatgtggccacactgcccctcaggaaggttctggctgtggtggggactgcggaggccagcagtgaacaccccttgggcgtggcagtcaccaaatactgtaaagaggaacttggaacagagaccttgggatactgcacggacttccaggcagtgccaggctgtggaattgggtgcaaagtcagcaacgtggaaggcatcctggcccacagtgagcgccctttgagtgcaccggccagtcacctgaatgaggctggcagccttcccgcagaaaaagatgcagtcccccagaccttctctgtgctgattggaaaccgtgagtggctgaggcgcaacggtttaaccatttctagcgatgtcagtgacgctatgacagaccacgagatgaaaggacagacagccatcctggtggctattgacggtgtgctctgtgggatgatcgcaatcgcagacgctgtcaagcaggaggctgccctggctgtgcacacgctgcagagcatgggtgtggacgtggttctgatcacgggggacaaccggaagacagccagagctattgccacccaggttggcatcaacaaagtctttgcagaggtgctgccttcgcacaaggtggccaaggtccaggagctccagaataaagggaagaaagtcgccatggtgggggatggggtcaatgactccccggccttggcccaggcagacatgggtgtggccattggcaccggcacggatgtggccatcgaggcagccgacgtcgtccttatcagaaatgatttgctggatgtggtggctagcattcacctttccaagaggactgtccgaaggatacgcatcaacctggtcctggcactgatttataacctggttgggatacccattgcagcaggtgtcttcatgcccatcggcattgtgctgcagccctggatgggctcagcggccatggcagcctcctctgtgtctgtggtgctctcatccctgcagctcaagtgctataagaagcctgacctggagaggtatgaggcacaggcgcatggccacatgaagcccctgacggcatcccaggtcagtgtgcacataggcatggatgacaggtggcgggactcccccagggccacaccatgggaccaggtcagctatgtcagccaggtgtcgctgtcctccctgacgtccgacaagccatctcggcacagcgctgcagcagacgatgatggggacaagtggtctctgctcctgaatggcagggatgaggagcagtacatctgagatccagacatgataagatacattgatgagtttggacaaaccacaactagaatgcagtgaaaaaaatgctttatttgtgaaatttgtgatgctattgctttatttgtaaccattataagctgcaataaacaagttaacaacaacaattgcattcattttatgtttcaggttcagggggaggtgtgggaggttttttagaggaacccctagtgatggagttggccactccctctctgcgcgctcgctcgctcactgaggccgcccgggcaaagcccgggcgtcgggcgacctttggtcgcccggcctcagtgagcgagcgagcgcgcagagagggagtggccaa

SEQ ID NO: 15 - DNA, 3603 bp, Artificial Sequence
  Description of artificial sequence: Del 1-3 ATP7B, codon-optimized
atgcccgagcaggaaagacagatcaccgccagagagggcgccagccggaagatcctgagcaagctgagcctgcccaccagagcctgggagcccgccatgaagaagtccttcgccttcgacaacgtgggctacgagggcggcctggacggactgggaccatcttctcaggtggccacaagcaccgtgcgcgacggagccgagggctccggaacagatcacagaagcagcagcagccacagccctggcagcccccctagaaatcaggtgcagggcacctgtagcaccaccctgatcgccattgccggcatgacatgcgccagctgcgtgcactctattgagggcatgatctcccagctggaaggcgtgcagcagatcagtgtgtctctggccgagggcaccgccacagtgctgtacaaccctagcgtgatcagccccgaagaactgagagccgccattgaggacatgggattcgaagccagcgtggtgtccgagagctgctccaccaaccctctgggcaatcacagcgccggcaacagcatggtgcagaccaccgacggcacccccaccagcgtgcaggaagtggccccacatacaggcagactgcccgccaatcacgcccccgatatcctggccaagagcccccagagtacaagagccgtggccccccagaagtgcttcctgcagatcaagggcatgacttgtgcctcttgtgtgtccaatatcgagcggaacctgcagaaagaggccggcgtgctgtctgtgctggtggctctgatggccggcaaggccgagatcaaatacgaccccgaagtgattcagcccctggaaatcgcccagtttatccaggacctgggctttgaagccgccgtgatggaagattacgccggctccgacggcaacatcgagctgaccatcaccggaatgacctgcgcctcctgtgtgcacaacattgagtccaagctgacccggaccaacggcatcacctacgcctctgtggctctggccacctccaaggccctcgtgaagttcgatcccgagatcatcggccccagggacatcatcaagatcatcgaagagatcggcttccacgccagcctggcccagaggaaccctaacgcccaccacctggaccacaagatggaaatcaagcagtggaagaaaagcttcctgtgcagcctggtgttcggcatccccgtgatggccctgatgatctacatgctgatccccagcaacgagccccaccagtccatggtgctggatcacaacatcatccccggcctgtctatcctgaacctgatcttcttcatcctgtgcaccttcgtgcagctgctgggcggctggtacttctacgtgcaggcctacaagtccctgcggcacagatccgccaacatggacgtgctgatcgtgctggccacatctatcgcctacgtgtactccctcgtgatcctggtggtggccgtggccgagaaagccgagagaagccctgtgaccttcttcgacaccccccctatgctgttcgtgtttatcgccctgggccggtggctggaacacctggccaaaagcaagaccagcgaggccctggctaagctgatgagtctgcaggccaccgaggccacagtcgtgaccctgggcgaggacaacctgatcatccgcgaggaacaggtgccaatggaactggtgcagcggggcgacatcgtgaaggtggtgcctggcggcaagttccccgtggacggaaaagtgctggaagggaataccatggccgacgagagcctgatcacaggcgaggccatgcccgtgaccaagaaacctggcagcacagtgatcgccggcagcatcaatgcccacggcagcgtgctgattaaggccacacacgtgggcaacgataccaccctggctcagattgtgaagctggtggaagaggcccagatgagcaaggcccccattcagcagctggctgaccggttcagcggctacttcgtgccctttatcatcatcatgagcaccctgacactggtcgtgtggatcgtgatcggctttatcgacttcggagtggtgcagagatacttccccaaccctaacaagcacatcagccagacagaagtgatcatcagattcgcctttcagaccagcatcaccgtgctgtgtatcgcctgcccctgtagcctgggactggccacacctaccgctgtgatggtgggaacaggcgtggccgctcagaacggcatcctgatcaaggggggcaagcctctggaaatggctcacaagatcaagaccgtgatgttcgacaagaccggcaccatcacccacggcgtgcccagagtgatgagagtgctgctgctgggggatgtggccaccctgcctctgagaaaggtgctggctgtcgtgggcacagccgaggctagctctgaacacccactgggagtggccgtgacaaagtactgcaaagaggaactgggcaccgaaaccctgggctactgcaccgactttcaggccgtgcctggctgtggcatcggctgcaaggtgtccaacgtggaaggcatcctggcccacagcgagaggccactgtctgcccctgccagccacctgaacgaggccggatctctgcccgccgaaaaggacgctgtgccccagaccttctctgtgctgattggcaacagagagtggctgcggcggaacggcctgaccatctcctccgatgtgtccgacgccatgaccgaccacgagatgaagggccagaccgccattctggtggccattgacggggtgctgtgcggcatgatcgcaatcgccgatgccgtgaaacaggaagcagcactggccgtgcacaccctgcagtctatgggagtggatgtggtgctgatcaccggcgacaacagaaagaccgccagggccattgccacccaggtgggcatcaacaaggtgttcgccgaggtgctgcccagccacaaagtggccaaggtgcaggaactgcagaacaaaggcaaaaaggtggccatggtgggagatggcgtgaacgactctcctgctctggcccaggcagatatgggcgtggccatcggcacaggcaccgacgtggcaattgaggctgctgacgtggtgctgattcggaacgacctgctggacgtggtggcctccatccacctgtccaagagaaccgtgcggcggatcagaatcaacctggtgctggcactgatctataacctcgtgggcatccctatcgccgctggcgtgttcatgcctatcggaatcgtgctgcagccctggatgggctctgccgccatggctgcaagctccgtgtctgtggtgctgtccagcctgcagctgaagtgctacaagaagcccgacctggaaagatacgaggcccaggcccacggacacatgaagcctctgacagcctcccaggtgtccgtgcacatcggcatggacgacagatggcgggacagccctagagccaccccttgggatcaggtgtcatacgtgtcacaggtgtccctgagcagcctgaccagcgacaagcccagcagacatagcgccgctgccgacgacgatggggacaagtggtccctgctgctgaacggccgggatgaggaacagtacatctga